European Patent Application EP 4 458 974 A1, published November 6, 2024. Title: Temperature sensitive minus-chain RNA virus and virus vector. Applicant: 株式会社レプリテック. The sequence listing filed with the application follows.

SEQUENCE LISTING (28 sequences)

SEQ ID NO: 1 - protein, 568 aa, Sendai virus
MDQDAFILKEDSEVEREAPGGRESLSDVIGFLDAVLSSEPTDIGGDRSWLHNTINTPQGPGSAHRAKSEGEGEVSTPSTQDNRSGEESRVSGRTSKPEAEAHAGNLDKQNIHRAFGGRTGTNSVSQDLGDGGDSGILENPPNERGYPRSGIEDENREMAAHPDKRGEDQAEGLPEEVRGSTSLPDEGEGGASNNGRSMEPGSSHSARVTGVLVIPSPELEEAVLRRNKRRPTNSGSKPLTPATVPGTRSPPLNRYNSTGSPPGKPPSTQDEHINSGDTPAVRVKDRKPPIGTRSVSDCPANGRPIHPGLETDSTKKGIGENTSSMKEMATLLTSLGVIQSAQEFESSRDASYVFARRALKSANYAEMTFNVCGLILSAEKSSARKVDENKQLLKQIQESVESFRDIYKRFSEYQKEQNSLLMSNLSTLHIITDRGGKTDNTDSLTRSPSVFAKSKENKTKATRFDPSMETLEDMKYKPDLIREDEFRDEIRNPVYQERDTEPRASNASRLLPSKEKPTMHSLRLVIESSPLSRAEKVAYVKSLSKCKTDQEVKAVMELVEEDIESLTN

SEQ ID NO: 2 - protein, 568 aa, synthetic construct
  REGION 1..568: note = Sendai virus Protein mutant P2
MDQDAFILKEDSEVEREAPGGRESLSDVIGFLDAVLSSEPTDIGGDRSWLHNTINTPQGPGSAHRAKSEGEGEVSTPSTQDNRSGEESRVSGRTSKPEAEAHAGNLDKQNIHRAFGGRTGTNSVSQDLGDGGDSGILENPPNERGYPRSGIEDENREMAAHPDKRGEDQAEGLPEEVRGSTSLPDEGEGGASNNGRSMEPGSSHSARVTGVLVIPSPELEEAVLRRNKRRPTNSGSKPLTPATVPGTRSPPLNRYNSTGSPPGKPPSTQDEHINSGDTPAVRVKDRKPPIGTRSVSDCPANGRPIHPGLETDSTKKGIGENTSSMKEMATLLTSLGVIQSAQEFESSRDASYVFARRALKSANYAEMTFNVCGLILSAEKSSARKVDENKQLLKQIQESVESFRDIYKRFSEYQKEQNSLLMSNLSTLHIITAAGGATDNTDSLTRSPSVFAKSKENKTKATRFDPSMETLEDMKYKPDLIREDEFRDEIRNPVYQERDTEPRASNASRLFPSKEKPTMHSLRLVIESSPLSRAEKVAYVKSLSKCKTDQEVKAVMELVEEDIESLTN

SEQ ID NO: 3 - protein, 568 aa, synthetic construct
  REGION 1..568: note = Sendai virus P protein L511F mutant
MDQDAFILKEDSEVEREAPGGRESLSDVIGFLDAVLSSEPTDIGGDRSWLHNTINTPQGPGSAHRAKSEGEGEVSTPSTQDNRSGEESRVSGRTSKPEAEAHAGNLDKQNIHRAFGGRTGTNSVSQDLGDGGDSGILENPPNERGYPRSGIEDENREMAAHPDKRGEDQAEGLPEEVRGSTSLPDEGEGGASNNGRSMEPGSSHSARVTGVLVIPSPELEEAVLRRNKRRPTNSGSKPLTPATVPGTRSPPLNRYNSTGSPPGKPPSTQDEHINSGDTPAVRVKDRKPPIGTRSVSDCPANGRPIHPGLETDSTKKGIGENTSSMKEMATLLTSLGVIQSAQEFESSRDASYVFARRALKSANYAEMTFNVCGLILSAEKSSARKVDENKQLLKQIQESVESFRDIYKRFSEYQKEQNSLLMSNLSTLHIITDRGGKTDNTDSLTRSPSVFAKSKENKTKATRFDPSMETLEDMKYKPDLIREDEFRDEIRNPVYQERDTEPRASNASRLFPSKEKPTMHSLRLVIESSPLSRAEKVAYVKSLSKCKTDQEVKAVMELVEEDIESLTN

SEQ ID NO: 4 - protein, 568 aa, synthetic construct
  REGION 1..568: note = Sendai virus P protein TS mutants
  SITE 433: note = MISC_FEATURE - X1 = any one of D, A, S, T, or G
  SITE 434: note = MISC_FEATURE - X2 = any one of R, A, S, T, or G
  SITE 437: note = MISC_FEATURE - X3 = any one of K, A, S, T, or G
  SITE 511: note = MISC_FEATURE - X3 = any one of L, F, or Y
MDQDAFILKEDSEVEREAPGGRESLSDVIGFLDAVLSSEPTDIGGDRSWLHNTINTPQGPGSAHRAKSEGEGEVSTPSTQDNRSGEESRVSGRTSKPEAEAHAGNLDKQNIHRAFGGRTGTNSVSQDLGDGGDSGILENPPNERGYPRSGIEDENREMAAHPDKRGEDQAEGLPEEVRGSTSLPDEGEGGASNNGRSMEPGSSHSARVTGVLVIPSPELEEAVLRRNKRRPTNSGSKPLTPATVPGTRSPPLNRYNSTGSPPGKPPSTQDEHINSGDTPAVRVKDRKPPIGTRSVSDCPANGRPIHPGLETDSTKKGIGENTSSMKEMATLLTSLGVIQSAQEFESSRDASYVFARRALKSANYAEMTFNVCGLILSAEKSSARKVDENKQLLKQIQESVESFRDIYKRFSEYQKEQNSLLMSNLSTLHIITXXGGXTDNTDSLTRSPSVFAKSKENKTKATRFDPSMETLEDMKYKPDLIREDEFRDEIRNPVYQERDTEPRASNASRLXPSKEKPTMHSLRLVIESSPLSRAEKVAYVKSLSKCKTDQEVKAVMELVEEDIESLTN

SEQ ID NO: 5 - protein, 2228 aa, Sendai virus
MDGQESSQNPSDILYPECHLNSPIVRGKIAQLHVLLDVNQPYRLKDDSIINITKHKIRNGGLSPRQIKIRSLGKALQRTIKDLDRYTFEPYPTYSQELLRLDIPEICDKIRSVFAVSDRLTRELSSGFQDLWLNIFKQLGNIEGREGYDPLQDIGTIPEITDKYSRNRWYRPFLTWFSIKYDMRWMQKTRPGGPLDTSNSHNLLECKSYTLVTYGDLVMILNKLTLTGYILTPELVLMYCDVVEGRWNMSAAGHLDKKSIGITSKGEELWELVDSLFSSLGEEIYNVIALLEPLSLALIQLNDPVIPLRGAFMRHVLTELQTVLTSRDVYTDAEADTIVESLLAIFHGTSIDEKAEIFSFFRTFGHPSLEAVTAADKVRAHMYAQKAIKLKTLYECHAVFCTIIINGYRERHGGQWPPCDFPDHVCLELRNAQGSNTAISYECAVDNYTSFIGFKFRKFIEPQLDEDLTIYMKDKALSPRKEAWDSVYPDSNLYYKAPESEETRRLIEVFINDENFNPEEIINYVESGDWLKDEEFNISYSLKEKEIKQEGRLFAKMTYKMRAVQVLAETLLAKGIGELFSENGMVKGEIDLLKRLTTLSVSGVPRTDSVYNNSKSSEKRNEGMENKNSGGYWDEKKRSRHEFKATDSSTDGYETLSCFLTTDLKKYCLNWRFESTALFGQRCNEIFGFKTFFNWMHPVLERCTIYVGDPYCPVADRMHRQLQDHADSGIFIHNPRGGIEGYCQKLWTLISISAIHLAAVRVGVRVSAMVQGDNQAIAVTSRVPVAQTYKQKKNHVYEEITKYFGALRHVMFDVGHELKLNETIISSKMFVYSKRIYYDGKILPQCLKALTKCVFWSETLVDENRSACSNISTSIAKAIENGYSPILGYCIALYKTCQQVCISLGMTINPTISPTVRDQYFKGKNWLRCAVLIPANVGGFNYMSTSRCFVRNIGDPAVAALADLKRFIRADLLDKQVLYRVMNQEPGDSSFLDWASDPYSCNLPHSQSITTIIKNITARSVLQESPNPLLSGLFTETSGEEDLNLASFLMDRKVILPRVAHEILGNSLTGVREAIAGMLDTTKSLVRASVRKGGLSYGILRRLVNYDLLQYETLTRTLRKPVKDNIEYEYMCSVELAVGLRQKMWIHLTYGRPIHGLETPDPLELLRGIFIEGSEVCKLCRSEGADPIYTWFYLPDNIDLDTLTNGCPAIRIPYFGSATDERSEAQLGYVRNLSKPAKAAIRIAMVYTWAYGTDEISWMEAALIAQTRANLSLENLKLLTPVSTSTNLSHRLKDTATQMKFSSATLVRASRFITISNDNMALKEAGESKDTNLVYQQIMLTGLSLFEFNMRYKKGSLGKPLILHLHLNNGCCIMESPQEANIPPRSTLDLEITQENNKLIYDPDPLKDVDLELFSKVRDVVHTVDMTYWSDDEVIRATSICTAMTIADTMSQLDRDNLKEMIALVNDDDVNSLITEFMVIDVPLFCSTFGGILVNQFAYSLYGLNIRGREEIWGHVVRILKDTSHAVLKVLSNALSHPKIFKRFWNAGVVEPVYGPNLSNQDKILLALSVCEYSVDLFMHDWQGGVPLEIFICDNDPDVADMRRSSFLARHLAYLCSLAEISRDGPRLESMNSLERLESLKSYLELTFLDDPVLRYSQLTGLVIKVFPSTLTYIRKSSIKVLRTRGIGVPEVLEDWDPEADNALLDGIAAEIQQNIPLGHQTRAPFWGLRVSKSQVLRLRGYKEITRGEIGRSGVGLTLPFDGRYLSHQLRLFGINSTSCLKALELTYLLSPLVDKDKDRLYLGEGAGAMLSCYDATLGPCINYYNSGVYSCDVNGQRELNIYPAEVALVGKKLNNVTSLGQRVKVLFNGNPGSTWIGNDECEALIWNELQNSSIGLVHCDMEGGDHKDDQVVLHEHYSVIRIAYLVGDRDVVLISKIAPRLGTDWTRQLSLYLRYWDEVNLIVLKTSNPASTEMYLLSRHPKSDIIEDSKTVLASLLPLSKEDSIKIEKWILIEKAKAHEWVTRELREGSSSSGMLRPYHQALQTFGFEPNLYKLSRDFLSTMNIADTHNCMIAFNRVLKDTIFEWARITESDKRLKLTGKYDLYPVRDSGKLKTISRRLVLSWISLSMSTRLVTGSFPDQKFEARLQLGIVSLSSREIRNLRVITKTLLDRFEDIIHSITYRFLTKEIKILMKILGAVKMFGARQNEYTTVIDDGSLGDIEPYDSS

SEQ ID NO: 6 - protein, 2228 aa, synthetic construct
  REGION 1..2228: note = Sendai virus L protein mutants
  SITE 1197: note = MISC_FEATURE - X1 = N or S
  SITE 1361: note = MISC_FEATURE - X2 = L or C
  SITE 1558: note = MISC_FEATURE - X3 = L or I
  SITE 1796: note = MISC_FEATURE - X4 = K or E
MDGQESSQNPSDILYPECHLNSPIVRGKIAQLHVLLDVNQPYRLKDDSIINITKHKIRNGGLSPRQIKIRSLGKALQRTIKDLDRYTFEPYPTYSQELLRLDIPEICDKIRSVFAVSDRLTRELSSGFQDLWLNIFKQLGNIEGREGYDPLQDIGTIPEITDKYSRNRWYRPFLTWFSIKYDMRWMQKTRPGGPLDTSNSHNLLECKSYTLVTYGDLVMILNKLTLTGYILTPELVLMYCDVVEGRWNMSAAGHLDKKSIGITSKGEELWELVDSLFSSLGEEIYNVIALLEPLSLALIQLNDPVIPLRGAFMRHVLTELQTVLTSRDVYTDAEADTIVESLLAIFHGTSIDEKAEIFSFFRTFGHPSLEAVTAADKVRAHMYAQKAIKLKTLYECHAVFCTIIINGYRERHGGQWPPCDFPDHVCLELRNAQGSNTAISYECAVDNYTSFIGFKFRKFIEPQLDEDLTIYMKDKALSPRKEAWDSVYPDSNLYYKAPESEETRRLIEVFINDENFNPEEIINYVESGDWLKDEEFNISYSLKEKEIKQEGRLFAKMTYKMRAVQVLAETLLAKGIGELFSENGMVKGEIDLLKRLTTLSVSGVPRTDSVYNNSKSSEKRNEGMENKNSGGYWDEKKRSRHEFKATDSSTDGYETLSCFLTTDLKKYCLNWRFESTALFGQRCNEIFGFKTFFNWMHPVLERCTIYVGDPYCPVADRMHRQLQDHADSGIFIHNPRGGIEGYCQKLWTLISISAIHLAAVRVGVRVSAMVQGDNQAIAVTSRVPVAQTYKQKKNHVYEEITKYFGALRHVMFDVGHELKLNETIISSKMFVYSKRIYYDGKILPQCLKALTKCVFWSETLVDENRSACSNISTSIAKAIENGYSPILGYCIALYKTCQQVCISLGMTINPTISPTVRDQYFKGKNWLRCAVLIPANVGGFNYMSTSRCFVRNIGDPAVAALADLKRFIRADLLDKQVLYRVMNQEPGDSSFLDWASDPYSCNLPHSQSITTIIKNITARSVLQESPNPLLSGLFTETSGEEDLNLASFLMDRKVILPRVAHEILGNSLTGVREAIAGMLDTTKSLVRASVRKGGLSYGILRRLVNYDLLQYETLTRTLRKPVKDNIEYEYMCSVELAVGLRQKMWIHLTYGRPIHGLETPDPLELLRGIFIEGSEVCKLCRSEGADPIYTWFYLPDXIDLDTLTNGCPAIRIPYFGSATDERSEAQLGYVRNLSKPAKAAIRIAMVYTWAYGTDEISWMEAALIAQTRANLSLENLKLLTPVSTSTNLSHRLKDTATQMKFSSATLVRASRFITISNDNMALKEAGESKDTNLVYQQIMLTGLSLFEFNMRYKKGSLGKPXILHLHLNNGCCIMESPQEANIPPRSTLDLEITQENNKLIYDPDPLKDVDLELFSKVRDVVHTVDMTYWSDDEVIRATSICTAMTIADTMSQLDRDNLKEMIALVNDDDVNSLITEFMVIDVPLFCSTFGGILVNQFAYSLYGLNIRGREEIWGHVVRILKDTSHAVLKVLSNALSHPKIFKRFWNAGVVEPVYGPNXSNQDKILLALSVCEYSVDLFMHDWQGGVPLEIFICDNDPDVADMRRSSFLARHLAYLCSLAEISRDGPRLESMNSLERLESLKSYLELTFLDDPVLRYSQLTGLVIKVFPSTLTYIRKSSIKVLRTRGIGVPEVLEDWDPEADNALLDGIAAEIQQNIPLGHQTRAPFWGLRVSKSQVLRLRGYKEITRGEIGRSGVGLTLPFDGRYLSHQLRLFGINSTSCLKALELTYLLSPLVDXDKDRLYLGEGAGAMLSCYDATLGPCINYYNSGVYSCDVNGQRELNIYPAEVALVGKKLNNVTSLGQRVKVLFNGNPGSTWIGNDECEALIWNELQNSSIGLVHCDMEGGDHKDDQVVLHEHYSVIRIAYLVGDRDVVLISKIAPRLGTDWTRQLSLYLRYWDEVNLIVLKTSNPASTEMYLLSRHPKSDIIEDSKTVLASLLPLSKEDSIKIEKWILIEKAKAHEWVTRELREGSSSSGMLRPYHQALQTFGFEPNLYKLSRDFLSTMNIADTHNCMIAFNRVLKDTIFEWARITESDKRLKLTGKYDLYPVRDSGKLKTISRRLVLSWISLSMSTRLVTGSFPDQKFEARLQLGIVSLSSREIRNLRVITKTLLDRFEDIIHSITYRFLTKEIKILMKILGAVKMFGARQNEYTTVIDDGSLGDIEPYDSS

SEQ ID NO: 7 - protein, 2228 aa, synthetic construct
  REGION 1..2228: note = Sendai virus L protein N1197S/L1558I/K1796E mutant
MDGQESSQNPSDILYPECHLNSPIVRGKIAQLHVLLDVNQPYRLKDDSIINITKHKIRNGGLSPRQIKIRSLGKALQRTIKDLDRYTFEPYPTYSQELLRLDIPEICDKIRSVFAVSDRLTRELSSGFQDLWLNIFKQLGNIEGREGYDPLQDIGTIPEITDKYSRNRWYRPFLTWFSIKYDMRWMQKTRPGGPLDTSNSHNLLECKSYTLVTYGDLVMILNKLTLTGYILTPELVLMYCDVVEGRWNMSAAGHLDKKSIGITSKGEELWELVDSLFSSLGEEIYNVIALLEPLSLALIQLNDPVIPLRGAFMRHVLTELQTVLTSRDVYTDAEADTIVESLLAIFHGTSIDEKAEIFSFFRTFGHPSLEAVTAADKVRAHMYAQKAIKLKTLYECHAVFCTIIINGYRERHGGQWPPCDFPDHVCLELRNAQGSNTAISYECAVDNYTSFIGFKFRKFIEPQLDEDLTIYMKDKALSPRKEAWDSVYPDSNLYYKAPESEETRRLIEVFINDENFNPEEIINYVESGDWLKDEEFNISYSLKEKEIKQEGRLFAKMTYKMRAVQVLAETLLAKGIGELFSENGMVKGEIDLLKRLTTLSVSGVPRTDSVYNNSKSSEKRNEGMENKNSGGYWDEKKRSRHEFKATDSSTDGYETLSCFLTTDLKKYCLNWRFESTALFGQRCNEIFGFKTFFNWMHPVLERCTIYVGDPYCPVADRMHRQLQDHADSGIFIHNPRGGIEGYCQKLWTLISISAIHLAAVRVGVRVSAMVQGDNQAIAVTSRVPVAQTYKQKKNHVYEEITKYFGALRHVMFDVGHELKLNETIISSKMFVYSKRIYYDGKILPQCLKALTKCVFWSETLVDENRSACSNISTSIAKAIENGYSPILGYCIALYKTCQQVCISLGMTINPTISPTVRDQYFKGKNWLRCAVLIPANVGGFNYMSTSRCFVRNIGDPAVAALADLKRFIRADLLDKQVLYRVMNQEPGDSSFLDWASDPYSCNLPHSQSITTIIKNITARSVLQESPNPLLSGLFTETSGEEDLNLASFLMDRKVILPRVAHEILGNSLTGVREAIAGMLDTTKSLVRASVRKGGLSYGILRRLVNYDLLQYETLTRTLRKPVKDNIEYEYMCSVELAVGLRQKMWIHLTYGRPIHGLETPDPLELLRGIFIEGSEVCKLCRSEGADPIYTWFYLPDSIDLDTLTNGCPAIRIPYFGSATDERSEAQLGYVRNLSKPAKAAIRIAMVYTWAYGTDEISWMEAALIAQTRANLSLENLKLLTPVSTSTNLSHRLKDTATQMKFSSATLVRASRFITISNDNMALKEAGESKDTNLVYQQIMLTGLSLFEFNMRYKKGSLGKPLILHLHLNNGCCIMESPQEANIPPRSTLDLEITQENNKLIYDPDPLKDVDLELFSKVRDVVHTVDMTYWSDDEVIRATSICTAMTIADTMSQLDRDNLKEMIALVNDDDVNSLITEFMVIDVPLFCSTFGGILVNQFAYSLYGLNIRGREEIWGHVVRILKDTSHAVLKVLSNALSHPKIFKRFWNAGVVEPVYGPNISNQDKILLALSVCEYSVDLFMHDWQGGVPLEIFICDNDPDVADMRRSSFLARHLAYLCSLAEISRDGPRLESMNSLERLESLKSYLELTFLDDPVLRYSQLTGLVIKVFPSTLTYIRKSSIKVLRTRGIGVPEVLEDWDPEADNALLDGIAAEIQQNIPLGHQTRAPFWGLRVSKSQVLRLRGYKEITRGEIGRSGVGLTLPFDGRYLSHQLRLFGINSTSCLKALELTYLLSPLVDEDKDRLYLGEGAGAMLSCYDATLGPCINYYNSGVYSCDVNGQRELNIYPAEVALVGKKLNNVTSLGQRVKVLFNGNPGSTWIGNDECEALIWNELQNSSIGLVHCDMEGGDHKDDQVVLHEHYSVIRIAYLVGDRDVVLISKIAPRLGTDWTRQLSLYLRYWDEVNLIVLKTSNPASTEMYLLSRHPKSDIIEDSKTVLASLLPLSKEDSIKIEKWILIEKAKAHEWVTRELREGSSSSGMLRPYHQALQTFGFEPNLYKLSRDFLSTMNIADTHNCMIAFNRVLKDTIFEWARITESDKRLKLTGKYDLYPVRDSGKLKTISRRLVLSWISLSMSTRLVTGSFPDQKFEARLQLGIVSLSSREIRNLRVITKTLLDRFEDIIHSITYRFLTKEIKILMKILGAVKMFGARQNEYTTVIDDGSLGDIEPYDSS

SEQ ID NO: 8 - protein, 568 aa, synthetic construct
  REGION 1..568: note = P2Y
MDQDAFILKEDSEVEREAPGGRESLSDVIGFLDAVLSSEPTDIGGDRSWLHNTINTPQGPGSAHRAKSEGEGEVSTPSTQDNRSGEESRVSGRTSKPEAEAHAGNLDKQNIHRAFGGRTGTNSVSQDLGDGGDSGILENPPNERGYPRSGIEDENREMAAHPDKRGEDQAEGLPEEVRGSTSLPDEGEGGASNNGRSMEPGSSHSARVTGVLVIPSPELEEAVLRRNKRRPTNSGSKPLTPATVPGTRSPPLNRYNSTGSPPGKPPSTQDEHINSGDTPAVRVKDRKPPIGTRSVSDCPANGRPIHPGLETDSTKKGIGENTSSMKEMATLLTSLGVIQSAQEFESSRDASYVFARRALKSANYAEMTFNVCGLILSAEKSSARKVDENKQLLKQIQESVESFRDIYKRFSEYQKEQNSLLMSNLSTLHIITAAGGATDNTDSLTRSPSVFAKSKENKTKATRFDPSMETLEDMKYKPDLIREDEFRDEIRNPVYQERDTEPRASNASRLYPSKEKPTMHSLRLVIESSPLSRAEKVAYVKSLSKCKTDQEVKAVMELVEEDIESLTN

SEQ ID NO: 9 - protein, 568 aa, synthetic construct
  REGION 1..568: note = P2m3SY
MDQDAFILKEDSEVEREAPGGRESLSDVIGFLDAVLSSEPTDIGGDRSWLHNTINTPQGPGSAHRAKSEGEGEVSTPSTQDNRSGEESRVSGRTSKPEAEAHAGNLDKQNIHRAFGGRTGTNSVSQDLGDGGDSGILENPPNERGYPRSGIEDENREMAAHPDKRGEDQAEGLPEEVRGSTSLPDEGEGGASNNGRSMEPGSSHSARVTGVLVIPSPELEEAVLRRNKRRPTNSGSKPLTPATVPGTRSPPLNRYNSTGSPPGKPPSTQDEHINSGDTPAVRVKDRKPPIGTRSVSDCPANGRPIHPGLETDSTKKGIGENTSSMKEMATLLTSLGVIQSAQEFESSRDASYVFARRALKSANYAEMTFNVCGLILSAEKSSARKVDENKQLLKQIQESVESFRDIYKRFSEYQKEQNSLLMSNLSTLHIITSSGGSTDNTDSLTRSPSVFAKSKENKTKATRFDPSMETLEDMKYKPDLIREDEFRDEIRNPVYQERDTEPRASNASRLYPSKEKPTMHSLRLVIESSPLSRAEKVAYVKSLSKCKTDQEVKAVMELVEEDIESLTN

SEQ ID NO: 10 - protein, 568 aa, synthetic construct
  REGION 1..568: note = P2m3TY
MDQDAFILKEDSEVEREAPGGRESLSDVIGFLDAVLSSEPTDIGGDRSWLHNTINTPQGPGSAHRAKSEGEGEVSTPSTQDNRSGEESRVSGRTSKPEAEAHAGNLDKQNIHRAFGGRTGTNSVSQDLGDGGDSGILENPPNERGYPRSGIEDENREMAAHPDKRGEDQAEGLPEEVRGSTSLPDEGEGGASNNGRSMEPGSSHSARVTGVLVIPSPELEEAVLRRNKRRPTNSGSKPLTPATVPGTRSPPLNRYNSTGSPPGKPPSTQDEHINSGDTPAVRVKDRKPPIGTRSVSDCPANGRPIHPGLETDSTKKGIGENTSSMKEMATLLTSLGVIQSAQEFESSRDASYVFARRALKSANYAEMTFNVCGLILSAEKSSARKVDENKQLLKQIQESVESFRDIYKRFSEYQKEQNSLLMSNLSTLHIITTTGGTTDNTDSLTRSPSVFAKSKENKTKATRFDPSMETLEDMKYKPDLIREDEFRDEIRNPVYQERDTEPRASNASRLYPSKEKPTMHSLRLVIESSPLSRAEKVAYVKSLSKCKTDQEVKAVMELVEEDIESLTN

SEQ ID NO: 11 - protein, 568 aa, synthetic construct
  REGION 1..568: note = P2m3GY
MDQDAFILKEDSEVEREAPGGRESLSDVIGFLDAVLSSEPTDIGGDRSWLHNTINTPQGPGSAHRAKSEGEGEVSTPSTQDNRSGEESRVSGRTSKPEAEAHAGNLDKQNIHRAFGGRTGTNSVSQDLGDGGDSGILENPPNERGYPRSGIEDENREMAAHPDKRGEDQAEGLPEEVRGSTSLPDEGEGGASNNGRSMEPGSSHSARVTGVLVIPSPELEEAVLRRNKRRPTNSGSKPLTPATVPGTRSPPLNRYNSTGSPPGKPPSTQDEHINSGDTPAVRVKDRKPPIGTRSVSDCPANGRPIHPGLETDSTKKGIGENTSSMKEMATLLTSLGVIQSAQEFESSRDASYVFARRALKSANYAEMTFNVCGLILSAEKSSARKVDENKQLLKQIQESVESFRDIYKRFSEYQKEQNSLLMSNLSTLHIITGGGGGTDNTDSLTRSPSVFAKSKENKTKATRFDPSMETLEDMKYKPDLIREDEFRDEIRNPVYQERDTEPRASNASRLYPSKEKPTMHSLRLVIESSPLSRAEKVAYVKSLSKCKTDQEVKAVMELVEEDIESLTN

SEQ ID NO: 12 - protein, 568 aa, synthetic construct
  REGION 1..568: note = P2m3SF
MDQDAFILKEDSEVEREAPGGRESLSDVIGFLDAVLSSEPTDIGGDRSWLHNTINTPQGPGSAHRAKSEGEGEVSTPSTQDNRSGEESRVSGRTSKPEAEAHAGNLDKQNIHRAFGGRTGTNSVSQDLGDGGDSGILENPPNERGYPRSGIEDENREMAAHPDKRGEDQAEGLPEEVRGSTSLPDEGEGGASNNGRSMEPGSSHSARVTGVLVIPSPELEEAVLRRNKRRPTNSGSKPLTPATVPGTRSPPLNRYNSTGSPPGKPPSTQDEHINSGDTPAVRVKDRKPPIGTRSVSDCPANGRPIHPGLETDSTKKGIGENTSSMKEMATLLTSLGVIQSAQEFESSRDASYVFARRALKSANYAEMTFNVCGLILSAEKSSARKVDENKQLLKQIQESVESFRDIYKRFSEYQKEQNSLLMSNLSTLHIITSSGGSTDNTDSLTRSPSVFAKSKENKTKATRFDPSMETLEDMKYKPDLIREDEFRDEIRNPVYQERDTEPRASNASRLFPSKEKPTMHSLRLVIESSPLSRAEKVAYVKSLSKCKTDQEVKAVMELVEEDIESLTN

SEQ ID NO: 13 - protein, 568 aa, synthetic construct
  REGION 1..568: note = P2m433S
MDQDAFILKEDSEVEREAPGGRESLSDVIGFLDAVLSSEPTDIGGDRSWLHNTINTPQGPGSAHRAKSEGEGEVSTPSTQDNRSGEESRVSGRTSKPEAEAHAGNLDKQNIHRAFGGRTGTNSVSQDLGDGGDSGILENPPNERGYPRSGIEDENREMAAHPDKRGEDQAEGLPEEVRGSTSLPDEGEGGASNNGRSMEPGSSHSARVTGVLVIPSPELEEAVLRRNKRRPTNSGSKPLTPATVPGTRSPPLNRYNSTGSPPGKPPSTQDEHINSGDTPAVRVKDRKPPIGTRSVSDCPANGRPIHPGLETDSTKKGIGENTSSMKEMATLLTSLGVIQSAQEFESSRDASYVFARRALKSANYAEMTFNVCGLILSAEKSSARKVDENKQLLKQIQESVESFRDIYKRFSEYQKEQNSLLMSNLSTLHIITSAGGATDNTDSLTRSPSVFAKSKENKTKATRFDPSMETLEDMKYKPDLIREDEFRDEIRNPVYQERDTEPRASNASRLFPSKEKPTMHSLRLVIESSPLSRAEKVAYVKSLSKCKTDQEVKAVMELVEEDIESLTN

SEQ ID NO: 14 - protein, 568 aa, synthetic construct
  REGION 1..568: note = P2m433SY
MDQDAFILKEDSEVEREAPGGRESLSDVIGFLDAVLSSEPTDIGGDRSWLHNTINTPQGPGSAHRAKSEGEGEVSTPSTQDNRSGEESRVSGRTSKPEAEAHAGNLDKQNIHRAFGGRTGTNSVSQDLGDGGDSGILENPPNERGYPRSGIEDENREMAAHPDKRGEDQAEGLPEEVRGSTSLPDEGEGGASNNGRSMEPGSSHSARVTGVLVIPSPELEEAVLRRNKRRPTNSGSKPLTPATVPGTRSPPLNRYNSTGSPPGKPPSTQDEHINSGDTPAVRVKDRKPPIGTRSVSDCPANGRPIHPGLETDSTKKGIGENTSSMKEMATLLTSLGVIQSAQEFESSRDASYVFARRALKSANYAEMTFNVCGLILSAEKSSARKVDENKQLLKQIQESVESFRDIYKRFSEYQKEQNSLLMSNLSTLHIITSAGGATDNTDSLTRSPSVFAKSKENKTKATRFDPSMETLEDMKYKPDLIREDEFRDEIRNPVYQERDTEPRASNASRLYPSKEKPTMHSLRLVIESSPLSRAEKVAYVKSLSKCKTDQEVKAVMELVEEDIESLTN

SEQ ID NO: 15 - protein, 568 aa, synthetic construct
  REGION 1..568: note = P2m434SY
MDQDAFILKEDSEVEREAPGGRESLSDVIGFLDAVLSSEPTDIGGDRSWLHNTINTPQGPGSAHRAKSEGEGEVSTPSTQDNRSGEESRVSGRTSKPEAEAHAGNLDKQNIHRAFGGRTGTNSVSQDLGDGGDSGILENPPNERGYPRSGIEDENREMAAHPDKRGEDQAEGLPEEVRGSTSLPDEGEGGASNNGRSMEPGSSHSARVTGVLVIPSPELEEAVLRRNKRRPTNSGSKPLTPATVPGTRSPPLNRYNSTGSPPGKPPSTQDEHINSGDTPAVRVKDRKPPIGTRSVSDCPANGRPIHPGLETDSTKKGIGENTSSMKEMATLLTSLGVIQSAQEFESSRDASYVFARRALKSANYAEMTFNVCGLILSAEKSSARKVDENKQLLKQIQESVESFRDIYKRFSEYQKEQNSLLMSNLSTLHIITASGGATDNTDSLTRSPSVFAKSKENKTKATRFDPSMETLEDMKYKPDLIREDEFRDEIRNPVYQERDTEPRASNASRLYPSKEKPTMHSLRLVIESSPLSRAEKVAYVKSLSKCKTDQEVKAVMELVEEDIESLTN

SEQ ID NO: 16 - protein, 568 aa, synthetic construct
  REGION 1..568: note = P2m437SY
MDQDAFILKEDSEVEREAPGGRESLSDVIGFLDAVLSSEPTDIGGDRSWLHNTINTPQGPGSAHRAKSEGEGEVSTPSTQDNRSGEESRVSGRTSKPEAEAHAGNLDKQNIHRAFGGRTGTNSVSQDLGDGGDSGILENPPNERGYPRSGIEDENREMAAHPDKRGEDQAEGLPEEVRGSTSLPDEGEGGASNNGRSMEPGSSHSARVTGVLVIPSPELEEAVLRRNKRRPTNSGSKPLTPATVPGTRSPPLNRYNSTGSPPGKPPSTQDEHINSGDTPAVRVKDRKPPIGTRSVSDCPANGRPIHPGLETDSTKKGIGENTSSMKEMATLLTSLGVIQSAQEFESSRDASYVFARRALKSANYAEMTFNVCGLILSAEKSSARKVDENKQLLKQIQESVESFRDIYKRFSEYQKEQNSLLMSNLSTLHIITAAGGSTDNTDSLTRSPSVFAKSKENKTKATRFDPSMETLEDMKYKPDLIREDEFRDEIRNPVYQERDTEPRASNASRLYPSKEKPTMHSLRLVIESSPLSRAEKVAYVKSLSKCKTDQEVKAVMELVEEDIESLTN

SEQ ID NO: 17 - protein, 2228 aa, synthetic construct
  REGION 1..2228: note = LmCI
MDGQESSQNPSDILYPECHLNSPIVRGKIAQLHVLLDVNQPYRLKDDSIINITKHKIRNGGLSPRQIKIRSLGKALQRTIKDLDRYTFEPYPTYSQELLRLDIPEICDKIRSVFAVSDRLTRELSSGFQDLWLNIFKQLGNIEGREGYDPLQDIGTIPEITDKYSRNRWYRPFLTWFSIKYDMRWMQKTRPGGPLDTSNSHNLLECKSYTLVTYGDLVMILNKLTLTGYILTPELVLMYCDVVEGRWNMSAAGHLDKKSIGITSKGEELWELVDSLFSSLGEEIYNVIALLEPLSLALIQLNDPVIPLRGAFMRHVLTELQTVLTSRDVYTDAEADTIVESLLAIFHGTSIDEKAEIFSFFRTFGHPSLEAVTAADKVRAHMYAQKAIKLKTLYECHAVFCTIIINGYRERHGGQWPPCDFPDHVCLELRNAQGSNTAISYECAVDNYTSFIGFKFRKFIEPQLDEDLTIYMKDKALSPRKEAWDSVYPDSNLYYKAPESEETRRLIEVFINDENFNPEEIINYVESGDWLKDEEFNISYSLKEKEIKQEGRLFAKMTYKMRAVQVLAETLLAKGIGELFSENGMVKGEIDLLKRLTTLSVSGVPRTDSVYNNSKSSEKRNEGMENKNSGGYWDEKKRSRHEFKATDSSTDGYETLSCFLTTDLKKYCLNWRFESTALFGQRCNEIFGFKTFFNWMHPVLERCTIYVGDPYCPVADRMHRQLQDHADSGIFIHNPRGGIEGYCQKLWTLISISAIHLAAVRVGVRVSAMVQGDNQAIAVTSRVPVAQTYKQKKNHVYEEITKYFGALRHVMFDVGHELKLNETIISSKMFVYSKRIYYDGKILPQCLKALTKCVFWSETLVDENRSACSNISTSIAKAIENGYSPILGYCIALYKTCQQVCISLGMTINPTISPTVRDQYFKGKNWLRCAVLIPANVGGFNYMSTSRCFVRNIGDPAVAALADLKRFIRADLLDKQVLYRVMNQEPGDSSFLDWASDPYSCNLPHSQSITTIIKNITARSVLQESPNPLLSGLFTETSGEEDLNLASFLMDRKVILPRVAHEILGNSLTGVREAIAGMLDTTKSLVRASVRKGGLSYGILRRLVNYDLLQYETLTRTLRKPVKDNIEYEYMCSVELAVGLRQKMWIHLTYGRPIHGLETPDPLELLRGIFIEGSEVCKLCRSEGADPIYTWFYLPDSIDLDTLTNGCPAIRIPYFGSATDERSEAQLGYVRNLSKPAKAAIRIAMVYTWAYGTDEISWMEAALIAQTRANLSLENLKLLTPVSTSTNLSHRLKDTATQMKFSSATLVRASRFITISNDNMALKEAGESKDTNLVYQQIMLTGLSLFEFNMRYKKGSLGKPCILHLHLNNGCCIMESPQEANIPPRSTLDLEITQENNKLIYDPDPLKDVDLELFSKVRDVVHTVDMTYWSDDEVIRATSICTAMTIADTMSQLDRDNLKEMIALVNDDDVNSLITEFMVIDVPLFCSTFGGILVNQFAYSLYGLNIRGREEIWGHVVRILKDTSHAVLKVLSNALSHPKIFKRFWNAGVVEPVYGPNISNQDKILLALSVCEYSVDLFMHDWQGGVPLEIFICDNDPDVADMRRSSFLARHLAYLCSLAEISRDGPRLESMNSLERLESLKSYLELTFLDDPVLRYSQLTGLVIKVFPSTLTYIRKSSIKVLRTRGIGVPEVLEDWDPEADNALLDGIAAEIQQNIPLGHQTRAPFWGLRVSKSQVLRLRGYKEITRGEIGRSGVGLTLPFDGRYLSHQLRLFGINSTSCLKALELTYLLSPLVDEDKDRLYLGEGAGAMLSCYDATLGPCINYYNSGVYSCDVNGQRELNIYPAEVALVGKKLNNVTSLGQRVKVLFNGNPGSTWIGNDECEALIWNELQNSSIGLVHCDMEGGDHKDDQVVLHEHYSVIRIAYLVGDRDVVLISKIAPRLGTDWTRQLSLYLRYWDEVNLIVLKTSNPASTEMYLLSRHPKSDIIEDSKTVLASLLPLSKEDSIKIEKWILIEKAKAHEWVTRELREGSSSSGMLRPYHQALQTFGFEPNLYKLSRDFLSTMNIADTHNCMIAFNRVLKDTIFEWARITESDKRLKLTGKYDLYPVRDSGKLKTISRRLVLSWISLSMSTRLVTGSFPDQKFEARLQLGIVSLSSREIRNLRVITKTLLDRFEDIIHSITYRFLTKEIKILMKILGAVKMFGARQNEYTTVIDDGSLGDIEPYDSS

SEQ ID NO: 18 - protein, 106 aa, synthetic construct
GVQVETISPGDGRTFPKRGQTCVVHYTGMLEDGKKVDSSRDRNKPFKFMLGKQEVIRGWEEGVAQMSVGQRAKLTISPDYAYGATGHPGIIPPHATLVFDVELLKP

SEQ ID NO: 19 - protein, 107 aa, synthetic construct
GVQIETISPGDGRTFPKKGQTCVVHYTGMLEDGKKLDSSRDRNKPFKFMIGKQEVIKGFEEGAAQMSLGQRAKLTISPDYAYGATGHPGVIPPHATLIFDVELLRPE

SEQ ID NO: 20 - protein, 348 aa, synthetic construct
MADIYRFPKFSYEDNGTVEPLPLRTGPDKKAIPHIRIVKVGDPPKHGVRYLDLLLLGFFETPKQTTNLESVSDLTEPTSYSICGSGSLPIGVAKYYGTDQELLKACTDLRITVRRAVRAGEMIVYMVDSIGAPLLPWSGRLRQGMIFNANKVALAPQCLPVDKDIRLRVVFVNGTSLGAITITKIPKTLADLALPNSISVNLLVTLKTGISTEQKGVLPVLDDQGEKKLNFMVHLGLIRRKVGKIYSVEYCKSKIERMRLIFSLGLIGGISFHVQVNGTLSKTFMSQLAWKRAVCFPLMDVNPHMNMVIWAASVEITGVDAVFQPAIPRDFRYYPNVVAKNIGRIRKL

SEQ ID NO: 21 - protein, 575 aa, synthetic construct
MDGDRGKRDSYWSTSPSGSTTKPASGWERSSKADTWLLILSFTQWALSIATVIICIIISARQGYSMKEYSMTVEALNMSSREVKESLTSLIRQEVIARAVNIQSSVQTGIPVLLNKNSRDVIQMIDKSCSRQELTQHCESTIAVHHADGIAPLEPHSFWRCPVGEPYLSSDPEISLLPGPSLLSGSTTISGCVRLPSLSIGEAIYAYSSNLITQGCADIGKSYQVLQLGYISLNSDMFPDLNPVVSHTYDINDNRKSCSVVTTKTRGYQLCSMPTVDERTDYSSDGIEDLVLDVLDLKGRTKSHRYRNSEVDLDHPFSALYPSVGNGIATEGSLIFLGYGGLTTPLQGDTKCRTQGCQQVSQDTCNEALKITWLGGKQVVSVIIQVNDYLSERPKIRVTTIPITQNYLGAEGRLLKLGDRVYIYTRSSGWHSQLQIGVLDVSHPLTINWTPHEALSRPGNEECNWYNKCPKECISGVYTDAYPLSPDAANVATVTLYANTSRVNPTIMYSNTTNIINMLRIKDVQLEAAYTTTSCITHFGKGYCFHIIEINQKSLNTLQPMLFKTSIPKLCKAES

SEQ ID NO: 22 - protein, 108 aa, Bos taurus
MGVQVETISPGDGRTFPKRGQTCVVHYTGMLEDGKKFDSSRDRNKPFKFVLGKQEVIRGWEEGVAQMSVGQRAKLTISPDYAYGATGHPGIIPPNATLIFDVELLKLE

SEQ ID NO: 23 - protein, 108 aa, Macaca mulatta
MGVEIETISPGDGRTFPKKGQTCVVHYTGMLQNGKKFDSSRDRNKPFKFRIGKQEVIKGFEEGAAQMSLGQRAKLTCTPDVAYGATGHPGVIPPNATLIFDVELLNLE

SEQ ID NO: 24 - protein, 108 aa, Homo sp.
MGVQVETISPGDGRTFPKRGQTCVVHYTGMLEDGKKFDSSRDRNKPFKFMLGKQEVIRGWEEGVAQMSVGQRAKLTISPDYAYGATGHPGIIPPHATLVFDVELLKLE

SEQ ID NO: 25 - protein, 108 aa, Mus musculus
MGVEIETISPGDGRTFPKKGQICVVHYTGMLQNGKKFDSSRDRNKPFKFRIGKQEVIKGFEEGTAQMSLGQRAKLTCTPDVAYGATGHPGVIPPNATLIFDVELLSLE

SEQ ID NO: 26 - protein, 108 aa, Oryctolagus cuniculus; identical to SEQ ID NO: 24

SEQ ID NO: 27 - protein, 108 aa, Rattus norvegicus
MGVEIETISPGDGRTFPKKGQICVVHYTGMLQNGKKFDSSRDRNKPFKFRIGKQEVIKGFEEGAAQMSLGQRAKLTCTPDVAYGATGHPGVIPPNATLIFDVELLNLE

SEQ ID NO: 28 - protein, 107 aa, synthetic construct
GVQVETISPGDGRTFPRRGQTCVVHYTGMLEDGRRVDSSRDRNRPFRFMLGRQEVIRGWEEGVSQMSVGQRSRLTISPDYSYGSTGHPGIIPPHSTLVFDVELLRPE